European Patent Application EP 4 349 969 A1, published April 10, 2024. Title: Composition for expanding natural killer cells comprising feeder cells. Applicant: Vaxcell-Bio KONGJU NATIONAL UNIVERSITY INDUSTRY-UNIVERSITY COOPERATION FOUNDATION. The sequence listing filed with the application follows.

SEQUENCE LISTING (4 sequences)

SEQ ID NO: 1 - DNA, 762 bp, Artificial Sequence
  B7H6
atggcgcacgggccgccgctcctgctcctgcccgcgctcctgctcctgccggcgctcctggtcctggtcctgtggttcgggacggccagctcaggtctcctgcaagtggagatggcagggaagactcagaaggtgctcctaaatgatactgccaccattgtctgcaaaatccatggttaccaccatctggacatcacagtaatgggtattacctggtattggaagcatcaggcctctgcaacggaagttaaactgtttgagttttttggtgaccatcaaatgatattacgatctggagcctacgtgtctcaaaggaggctgcaaaggggggatgcctccctccagctgccaggcgtccagctgaaggaagcaggagagtaccgatgtgaggtggtggtcaccccttacaaagcagtgggaacagtcaacctggaggttgtggcttaccccgtcagcagcttgtctccagagcaagccatggtgaaagaaaatgaagaacaacttattttgtgtatggcaagtaggttctaccccaagaacattaccataacatggaaaaagtggaccccaaaggatccccggtatctggaggtttctgagggcatcattactaatggtaccaccgaagatgaggatggcatgtttagtgtcactagttacttgatggtgaagccctctttggaagacaatatgactgtctatcagtgtgtggtatggcatgaatccttgccaatctcccagagccgcaacttcaccttgatt

SEQ ID NO: 2 - DNA, 774 bp, Artificial Sequence
  CD137L
atgcgcccccgcagcgacgccgccccggaccccgaggccccgcggccgcccgcgccccccggccgcacctgcagcccgctgccctgggcgctgagcgccgcgatgctgctgctcgtcggcacctgcgccgcctgcgcgctccgcgcctgggtggtccccgggccccggccccccgcgctccccgcgctccccgcgctccccgcgcccctgccggacgccggcgcccgcctccccgactccccgcaggccgtgttcgcgcagctggtggcccgagatgtacagctgaaggaaggacccctgcgctggtacagtgacccgggcctggcaggtgtattcctggggccgggcctgagttatgaccagcacactcgggagctgatggtggtggaacccgggctctactatgttttcttgcacctgaagctgcagcgggtaatgtccagcacgggctccggctctgtctctgctgccctgcacctgcagccacttggcaccgaggctgcagccctggacctgaccttggacctgcctccaccatcctcggaggcccgtgactcagcagctggtttccagggcagcctgctgcacctggacgcaggccagcgcctccgtgttcacttgcgagctgaggcaggggcccaccctgcctggcagctggcacaaggtgccacgatcttgggcctcttcagagtggccaccaaagtccccactggactcccctcgtcatggcccatggacacggggcctgggtccccgcccctggatggagaataa

SEQ ID NO: 3 - DNA, 342 bp, Artificial Sequence
  IL-15
aattggcaggacgtgatacttgatttggaaaaaattgacaatcttattcaatctatacatatggataccactctgtatactgaaagtgatgtgcatcccagttgcaaagtaaccgcgatgaagtgctttctcctggagttaggtgttatctcgctcgagtccggcagtcatcccattaaggaagcagtagagaacctcatcatcctcgcaaacagtgatctgtcttcgaaggggaatataactgaaacgggatgcaaagaatgtgaagaactggaggaaaagagtattaaggagtttttgcagagtttcgtgcatatcgtacaaatgttcatcaactcctct

SEQ ID NO: 4 - DNA, 597 bp, Artificial Sequence
  IL-15R alpha
atggcgcggacggggcggacggggccgccgctccggggccgccggctccccgcgctccccgcgctccccgcgctgctgctgctgctgctgccgctccggcccgcgacgccgggcatcacatgccctcctcccacatctgtcaaacacgcagatatccaggtcaagagttacagcgtgagctccaaggaacggtacacttgtaactctggcttcaagcggaaagccgggacatccagcctgactgagtgtgtgctcaacaagaccaccaacactgcccactggacaatccccagtctcaagtgcatcagagacccctccctgactcacctaaggccatcctcctcagacgtgccggcaggggtgaccccagagccagagagcacctccctttctggaaaagagccaactttcacttccaagtcagacaccaaagtggccacaaagccaactattgtgccaggctccaggccgatgccgtcaaagcctcctgctacaggaaccacagggctgatcagtaatgaaccctcctcccaagccccatctcagacaacagcaaaggccttggaacacactccctctgcctcccaggagacgcca